European Patent Application EP 4 177 606 A1, published May 10, 2023. Title: NANOPORE SYSTEM FOR SENSING USING IDENTIFICATION MOLECULES AND METHOD THEREOF. Applicant: IMEC VZW. Application EP 22204657.5, filed October 31, 2022. The sequence listing filed with the application follows.

SEQUENCE LISTING (2 sequences)

SEQ ID NO: 1 - DNA, 10 bp, synthetic construct
  source 1..10: mol_type = other DNA
acgttgaatt

SEQ ID NO: 2 - DNA, 10 bp, synthetic construct
  source 1..10: mol_type = other DNA
ccgtgaatcg